European Patent Specification EP 3 617 311 B1, published November 20, 2024. Title: METHOD FOR INDUCING EXON SKIPPING BY GENOME EDITING. Applicant: Kyoto University. The sequence listing filed with the application follows.

SEQUENCE LISTING (219 sequences)

SEQ ID NO: 1 - DNA, 20 bp, Artificial Sequence
  primer Luc2-Fwd-Splice
tgcccacactatttagcttc

SEQ ID NO: 2 - DNA, 20 bp, Artificial Sequence
  primer Luc2-Rev-Splice
gtcgatgagagcgtttgtag

SEQ ID NO: 3 - DNA, 83 bp, Artificial Sequence
  scaffold1
gttttagagctagaaatagcaagttaaaataaggctagtccgttatcaacttgaaaaagtggcaccgagtcggtgcttttttt

SEQ ID NO: 4 - DNA, 95 bp, Artificial Sequence
  modified scaffold
gttttagagctatgctggaaacagcatagcaagttaaaataaggctagtccgttatcaacttgaaaaagtggcaccgagtcggtgcttttttttt

SEQ ID NO: 5 - DNA, 21 bp, Artificial Sequence
  scaffold for Cpf1
gtaatttctactcttgtagat

SEQ ID NO: 6 - DNA, 23 bp, Artificial Sequence
  scaffold for Cpf1
gggtaatttctactcttgtagat

SEQ ID NO: 7 - DNA, 23 bp, Artificial Sequence
  spacer for Type II Cas9
  misc_feature (1)..(21): n is a, c, g, or t
nnnnnnnnnnnnnnnnnnnnngg

SEQ ID NO: 8 - DNA, 25 bp, Artificial Sequence
  Type V Cfp1 for Type V Cfp1
  misc_feature (6)..(25): n is a, c, g, or t
ttttvnnnnnnnnnnnnnnnnnnnn

SEQ ID NO: 9 - DNA, 20 bp, Artificial Sequence
  crRNA 1
tggtatcttacaggaactcc

SEQ ID NO: 10 - DNA, 20 bp, Artificial Sequence
  crRNA2
atcttacaggaactccagga

SEQ ID NO: 11 - DNA, 20 bp, Artificial Sequence
  crRNA3
caggaactccaggatggcat

SEQ ID NO: 12 - DNA, 20 bp, Artificial Sequence
  crRNA4
tccaggatggcattgggcag

SEQ ID NO: 13 - DNA, 20 bp, Artificial Sequence
  crRNA5
gttcctgtaagataccaaaa

SEQ ID NO: 14 - DNA, 275 bp, Artificial Sequence
  SphcCas9-D10A
attcagtcgaccatggataagaaatacagcattggactggccattgggacaaactccgtgggatgggccgtgattacagacgaatacaaagtgccttcaaagaagttcaaggtgctgggcaacaccgatagacacagcatcaagaaaaatctgattggagccctgctgttcgactccggcgagacagctgaagcaactcggctgaaaagaactgctcggagaaggtatacccgccgaaagaataggatctgctacctgcaggagattttcagcaa

SEQ ID NO: 15 - DNA, 135 bp, Artificial Sequence
  PCR product
  misc_feature (18)..(36): n is a, c, g, or t
gagaccacttggatccrnnnnnnnnnnnnnnnnnnngttttagagctagaaatagcaagttaaaataaggctagtccgttatcaacttgaaaaagtggcaccgagtcggtgctttttttgaattcaaacccgggc

SEQ ID NO: 16 - DNA, 57 bp, Artificial Sequence
  Sp-sgRNA-XXX-fwd
  misc_feature (18)..(36): n is a, c, g, or t
gagaccacttggatccrnnnnnnnnnnnnnnnnnnngttttagagctagaaatagca

SEQ ID NO: 17 - DNA, 57 bp, Artificial Sequence
  primer Sp-sgRNA-DMD1-fwd
gagaccacttggatccgggtatcttacaggaactccgttttagagctagaaatagca

SEQ ID NO: 18 - DNA, 57 bp, Artificial Sequence
  primer Sp-sgRNA-DMD2-fwd
gagaccacttggatccgtcttacaggaactccaggagttttagagctagaaatagca

SEQ ID NO: 19 - DNA, 57 bp, Artificial Sequence
  primer Sp-sgRNA-DMD3-fwd
gagaccacttggatccgaggaactccaggatggcatgttttagagctagaaatagca

SEQ ID NO: 20 - DNA, 57 bp, Artificial Sequence
  primer Sp-sgRNA-DMD4-fwd
gagaccacttggatccgccaggatggcattgggcaggttttagagctagaaatagca

SEQ ID NO: 21 - DNA, 57 bp, Artificial Sequence
  primer Sp-sgRNA-DMD5-fwd
gagaccacttggatccgttcctgtaagataccaaaagttttagagctagaaatagca

SEQ ID NO: 22 - DNA, 57 bp, Artificial Sequence
  primer Sp-sgRNA-DMD6-fwd
gagaccacttggatccgcatttttgttttgccttttgttttagagctagaaatagca

SEQ ID NO: 23 - DNA, 57 bp, Artificial Sequence
  primer Sp-sgRNA-DMD7fwd
gagaccacttggatccgtgcctttttggtatcttacgttttagagctagaaatagca

SEQ ID NO: 24 - DNA, 57 bp, Artificial Sequence
  primer Sp-sgRNA-DMD8-fwd
gagaccacttggatccaggaactccaggatggcattgttttagagctagaaatagca

SEQ ID NO: 25 - DNA, 57 bp, Artificial Sequence
  primer Sp-sgRNA-DMD9-fwd
gagaccacttggatccgccgctgcccaatgccatccgttttagagctagaaatagca

SEQ ID NO: 26 - DNA, 57 bp, Artificial Sequence
  primer Sp-sgRNA-DMD10-fwd
gagaccacttggatccgtcagaacattgaatgcaacgttttagagctagaaatagca

SEQ ID NO: 27 - DNA, 57 bp, Artificial Sequence
  primer Sp-sgRNA-DMD11-fwd
gagaccacttggatccgcagaacattgaatgcaactgttttagagctagaaatagca

SEQ ID NO: 28 - DNA, 57 bp, Artificial Sequence
  primer Sp-sgRNA-DMD12-fwd
gagaccacttggatccgagaacattgaatgcaactggttttagagctagaaatagca

SEQ ID NO: 29 - DNA, 57 bp, Artificial Sequence
  primer Sp-sgRNA-DMD13-fwd
gagaccacttggatccaatactggcatctgtttttggttttagagctagaaatagca

SEQ ID NO: 30 - DNA, 57 bp, Artificial Sequence
  primer Sp-sgRNA-DMD14-fwd
gagaccacttggatccaacagatgccagtattctacgttttagagctagaaatagca

SEQ ID NO: 31 - DNA, 57 bp, Artificial Sequence
  primer Sp-sgRNA-DMD15-fwd
gagaccacttggatccgaatttttcctgtagaatacgttttagagctagaaatagca

SEQ ID NO: 32 - DNA, 57 bp, Artificial Sequence
  primer Sp-sgRNA-DMD16-fwd
gagaccacttggatccgagtattctacaggaaaaatgttttagagctagaaatagca

SEQ ID NO: 33 - DNA, 57 bp, Artificial Sequence
  primer Sp-sgRNA-DMD17-fwd
gagaccacttggatccagtattctacaggaaaaattgttttagagctagaaatagca

SEQ ID NO: 34 - DNA, 57 bp, Artificial Sequence
  primer Sp-sgRNA-DMD18-fwd
gagaccacttggatccaattgggaagcctgaatctggttttagagctagaaatagca

SEQ ID NO: 35 - DNA, 57 bp, Artificial Sequence
  primer Sp-sgRNA-DMD19-fwd
gagaccacttggatccggggaagcctgaatctgcgggttttagagctagaaatagca

SEQ ID NO: 36 - DNA, 57 bp, Artificial Sequence
  primer Sp-sgRNA-DMD20-fwd
gagaccacttggatccaagcctgaatctgcggtggcgttttagagctagaaatagca

SEQ ID NO: 37 - DNA, 57 bp, Artificial Sequence
  primer Sp-sgRNA-DMD21-fwd
gagaccacttggatccgctgaatctgcggtggcagggttttagagctagaaatagca

SEQ ID NO: 38 - DNA, 57 bp, Artificial Sequence
  primer Sp-sgRNA-DMD22-fwd
gagaccacttggatccgctcctgccaccgcagattcgttttagagctagaaatagca

SEQ ID NO: 39 - DNA, 57 bp, Artificial Sequence
  primer Sp-sgRNA-DMD23-fwd
gagaccacttggatccagctgtcagacagaaaaaaggttttagagctagaaatagca

SEQ ID NO: 40 - DNA, 57 bp, Artificial Sequence
  primer Sp-sgRNA-DMD24-fwd
gagaccacttggatccgtcagacagaaaaaagaggtgttttagagctagaaatagca

SEQ ID NO: 41 - DNA, 57 bp, Artificial Sequence
  primer Sp-sgRNA-DMD25-fwd
gagaccacttggatccgcagacagaaaaaagaggtagttttagagctagaaatagca

SEQ ID NO: 42 - DNA, 57 bp, Artificial Sequence
  primer Sp-sgRNA-DMD26-fwd
gagaccacttggatccggtagggcgacagatctaatgttttagagctagaaatagca

SEQ ID NO: 43 - DNA, 96 bp, Artificial Sequence
  primer Sp-sgRNA-Universal-rev
gcccgggtttgaattcaaaaaaagcaccgactcggtgccactttttcaagttgataacggactagccttattttaacttgctatttctagctctaa

SEQ ID NO: 44 - DNA, 63 bp, Artificial Sequence
  primer sgRNA-DMD-SA-5
gagaccacttggatccattacaggaactccaggatggcagttttagtactctggaaacagaat

SEQ ID NO: 45 - DNA, 63 bp, Artificial Sequence
  primer sgRNA-DMD-SA-8
gagaccacttggatccattgccgctgcccaatgccatccgttttagtactctggaaacagaat

SEQ ID NO: 46 - DNA, 96 bp, Artificial Sequence
  primer SA1-gRNA-Universal-Rev
gcccgggtttgaattcaaaaaaatctcgccaacaagttgacgagataaacacggcattttgccttgttttagtagattctgtttccagagtactaa

SEQ ID NO: 47 - DNA, 39 bp, Artificial Sequence
  primer AsCpf1-gRNA-Universal-GGG-fwd
gagaccacttggatccgggtaatttctactcttgtagat

SEQ ID NO: 48 - DNA, 37 bp, Artificial Sequence
  primer AsCpf1-gRNA-Universal-G-fwd
gagaccacttggatccgtaatttctactcttgtagat

SEQ ID NO: 49 - DNA, 63 bp, Artificial Sequence
  primer AsCpf1-gRNA-XXX-rev
  misc_feature (24)..(43): n is a, c, g, or t
gcccgggtttgaattcaaaaaaannnnnnnnnnnnnnnnnnnnatctacaagagtagaaatta

SEQ ID NO: 50 - DNA, 63 bp, Artificial Sequence
  primer AsCpf1-gRNA-DMD1-rev
gcccgggtttgaattcaaaaaaaggagttcctgtaagataccaatctacaagagtagaaatta

SEQ ID NO: 51 - DNA, 63 bp, Artificial Sequence
  primer AsCpf1-gRNA-DMD2-rev
gcccgggtttgaattcaaaaaaatggagttcctgtaagataccatctacaagagtagaaatta

SEQ ID NO: 52 - DNA, 63 bp, Artificial Sequence
  primer AsCpf1-gRNA-DMD3-rev
gcccgggtttgaattcaaaaaaactggagttcctgtaagatacatctacaagagtagaaatta

SEQ ID NO: 53 - DNA, 63 bp, Artificial Sequence
  primer AsCpf1-gRNA-DMD4-rev
gcccgggtttgaattcaaaaaaaaggatggcattgggcagcggatctacaagagtagaaatta

SEQ ID NO: 54 - DNA, 74 bp, Artificial Sequence
  primer SSA-DMD-all-ss
gtcgtgcctttttggtatcttacaggaactccaggatggcattgggcagcggcaaactgttgtcagaacatggt

SEQ ID NO: 55 - DNA, 74 bp, Artificial Sequence
  primer SSA-DMD-all-as
cggtaccatgttctgacaacagtttgccgctgcccaatgccatcctggagttcctgtaagataccaaaaaggca

SEQ ID NO: 56 - DNA, 56 bp, Artificial Sequence
  primer DMD-MiSeq-Rd1-fwd-X
  misc_feature (31)..(34): n is a, c, g, or t
ctctttccctacacgacgctcttccgatctnnnnaataaaaagacatggggcttca

SEQ ID NO: 57 - DNA, 54 bp, Artificial Sequence
  primer DMD-MiSeq-Rd2-rev-X
  misc_feature (31)..(34): n is a, c, g, or t
ctggagttcagacgtgtgctcttccgatctnnnnctggcatctgtttttgagga

SEQ ID NO: 58 - DNA, 49 bp, Artificial Sequence
  primer Multiplex P5 fwd
aatgatacggcgaccaccgagatctacactctttccctacacgacgctc

SEQ ID NO: 59 - DNA, 49 bp, Artificial Sequence
  primer Multiplex P7 rev
caagcagaagacggcatacgagatgtgactggagttcagacgtgtgctc

SEQ ID NO: 60 - DNA, 56 bp, Artificial Sequence
  primer DMD-MiSeq-Rd1-fwd1-AGTC
ctctttccctacacgacgctcttccgatctagtcaataaaaagacatggggcttca

SEQ ID NO: 61 - DNA, 56 bp, Artificial Sequence
  primer DMD-MiSeq-Rd1-fwd2-GTCA
ctctttccctacacgacgctcttccgatctgtcaaataaaaagacatggggcttca

SEQ ID NO: 62 - DNA, 56 bp, Artificial Sequence
  primer DMD-MiSeq-Rd1-fwd3-TCAG
ctctttccctacacgacgctcttccgatcttcagaataaaaagacatggggcttca

SEQ ID NO: 63 - DNA, 56 bp, Artificial Sequence
  primer DMD-MiSeq-Rd1-fwd4-CAGT
ctctttccctacacgacgctcttccgatctcagtaataaaaagacatggggcttca

SEQ ID NO: 64 - DNA, 56 bp, Artificial Sequence
  primer DMD-MiSeq-Rd1-fwd5-ATGC
ctctttccctacacgacgctcttccgatctatgcaataaaaagacatggggcttca

SEQ ID NO: 65 - DNA, 56 bp, Artificial Sequence
  primer DMD-MiSeq-Rd1-fwd6-TGCA
ctctttccctacacgacgctcttccgatcttgcaaataaaaagacatggggcttca

SEQ ID NO: 66 - DNA, 56 bp, Artificial Sequence
  primer DMD-MiSeq-Rd1-fwd7-GCAT
ctctttccctacacgacgctcttccgatctgcataataaaaagacatggggcttca

SEQ ID NO: 67 - DNA, 56 bp, Artificial Sequence
  primer DMD-MiSeq-Rd1-fwd8-CATG
ctctttccctacacgacgctcttccgatctcatgaataaaaagacatggggcttca

SEQ ID NO: 68 - DNA, 56 bp, Artificial Sequence
  primer DMD-MiSeq-Rd1-fwd9-AACG
ctctttccctacacgacgctcttccgatctaacgaataaaaagacatggggcttca

SEQ ID NO: 69 - DNA, 56 bp, Artificial Sequence
  primer DMD-MiSeq-Rd1-fwd10-ACGA
ctctttccctacacgacgctcttccgatctacgaaataaaaagacatggggcttca

SEQ ID NO: 70 - DNA, 56 bp, Artificial Sequence
  primer DMD-MiSeq-Rd1-fwd11-CGAA
ctctttccctacacgacgctcttccgatctcgaaaataaaaagacatggggcttca

SEQ ID NO: 71 - DNA, 56 bp, Artificial Sequence
  primer DMD-MiSeq-Rd1-fwd12-GAAC
ctctttccctacacgacgctcttccgatctgaacaataaaaagacatggggcttca

SEQ ID NO: 72 - DNA, 56 bp, Artificial Sequence
  primer DMD-MiSeq-Rd1-fwd13-TACC
ctctttccctacacgacgctcttccgatcttaccaataaaaagacatggggcttca

SEQ ID NO: 73 - DNA, 56 bp, Artificial Sequence
  primer DMD-MiSeq-Rd1-fwd14-ACCT
ctctttccctacacgacgctcttccgatctacctaataaaaagacatggggcttca

SEQ ID NO: 74 - DNA, 54 bp, Artificial Sequence
  primer DMD-MiSeq-Rd2-rev1-AGTC
ctggagttcagacgtgtgctcttccgatctagtcctggcatctgtttttgagga

SEQ ID NO: 75 - DNA, 54 bp, Artificial Sequence
  primer DMD-MiSeq-Rd2-rev2-GTCA
ctggagttcagacgtgtgctcttccgatctgtcactggcatctgtttttgagga

SEQ ID NO: 76 - DNA, 54 bp, Artificial Sequence
  primer DMD-MiSeq-Rd2-rev3-TCAG
ctggagttcagacgtgtgctcttccgatcttcagctggcatctgtttttgagga

SEQ ID NO: 77 - DNA, 54 bp, Artificial Sequence
  primer DMD-MiSeq-Rd2-rev4-CAGT
ctggagttcagacgtgtgctcttccgatctcagtctggcatctgtttttgagga

SEQ ID NO: 78 - DNA, 54 bp, Artificial Sequence
  primer DMD-MiSeq-Rd2-rev5-ATGC
ctggagttcagacgtgtgctcttccgatctatgcctggcatctgtttttgagga

SEQ ID NO: 79 - DNA, 54 bp, Artificial Sequence
  primer DMD-MiSeq-Rd2-rev6-TGCA
ctggagttcagacgtgtgctcttccgatcttgcactggcatctgtttttgagga

SEQ ID NO: 80 - DNA, 54 bp, Artificial Sequence
  primer DMD-MiSeq-Rd2-rev7-GCAT
ctggagttcagacgtgtgctcttccgatctgcatctggcatctgtttttgagga

SEQ ID NO: 81 - DNA, 54 bp, Artificial Sequence
  primer DMD-MiSeq-Rd2-rev8-CATG
ctggagttcagacgtgtgctcttccgatctcatgctggcatctgtttttgagga

SEQ ID NO: 82 - DNA, 54 bp, Artificial Sequence
  primer DMD-MiSeq-Rd2-rev9-AACG
ctggagttcagacgtgtgctcttccgatctaacgctggcatctgtttttgagga

SEQ ID NO: 83 - DNA, 54 bp, Artificial Sequence
  primer DMD-MiSeq-Rd2-rev10-ACGA
ctggagttcagacgtgtgctcttccgatctacgactggcatctgtttttgagga

SEQ ID NO: 84 - DNA, 54 bp, Artificial Sequence
  primer DMD-MiSeq-Rd2-rev11-CGAA
ctggagttcagacgtgtgctcttccgatctcgaactggcatctgtttttgagga

SEQ ID NO: 85 - DNA, 54 bp, Artificial Sequence
  primer DMD-MiSeq-Rd2-rev12-GAAC
ctggagttcagacgtgtgctcttccgatctgaacctggcatctgtttttgagga

SEQ ID NO: 86 - DNA, 54 bp, Artificial Sequence
  primer DMD-MiSeq-Rd2-rev13-TACC
ctggagttcagacgtgtgctcttccgatcttaccctggcatctgtttttgagga

SEQ ID NO: 87 - DNA, 54 bp, Artificial Sequence
  primer DMD-MiSeq-Rd2-rev14-ACCT
ctggagttcagacgtgtgctcttccgatctacctctggcatctgtttttgagga

SEQ ID NO: 88 - DNA, 1000 bp, Artificial Sequence
  NarI-AgeI-DMD-Ex45-gBlock
gccagcggcggggcgccgctcagcaaggaggtaggtgaggccgtggccaaacgcttccacctaccaggtaagtctttgatttgtcgaccgtatccacgatcactaagaaacccaaatactttgttcatgtttaaattttacaacatttcatagactattaaacatggaacatccttgtggggacaagaaatcgaatttgctcttgaaaaggtttccaactaattgatttgtaggacattataacatcctctagctgacaagcttacaaaaataaaaactggagctaaccgagagggtgcttttttccctgacacataaaaggtgtctttctgtcttgtatcctttggatatgggcatgtcagtttcatagggaaattttcacatggagcttttgtatttctttctttgccagtacaactgcatgtggtagcacactgtttaatcttttctcaaataaaaagacatggggcttcatttttgttttgcctttttggtatcttacaggaactccaggatggcattgggcagcggcaaactgttgtcagaacattgaatgcaactggggaagaaataattcagcaatcctcaaaaacagatgccagtattctacaggaaaaattgggaagcctgaatctgcggtggcaggaggtctgcaaacagctgtcagacagaaaaaagaggtagggcgacagatctaataggaatgaaaacattttagcagactttttaagctttctttagaagaatatttcatgagagattataagcagggtgaaaggcgtcgacgtttgcattaacaaatagtttgagaactatgttggaaaaaaaaataacaattttattcttctttctccaggcatccgccagggctacggcctgacagaaacaaccagcgccattctgatcacccccgaaggggacgacaagcctggcgcagtaggcaaggtggtgcccttcttcgaggctaaggtggtggacttggacaccggtaagacactgg

SEQ ID NO: 89 - DNA, 396 bp, Artificial Sequence
  gBlock11-PV-3'TR-5'TR
gaaaagtgccacctgacgtcatctgttaacattatacgcgtttaaccctagaaagataatcatattgtgacgtacgttaaagataatcatgcgtaaaattgacgcatgtgttttatcggtctgtatatcgaggtttatttattaatttgaatagatattaagttttattatatttacacttacatactaataataaattcaacaaacaatttatttatgtttatttatttattaaaaaaaaacaaaaactcaaaatttcttctataaagtaacaaaacttttaaacattctctcttttacaaaaataaacttattttgtactttaaaaacagtcatgttgtattataaaataagtaattagcttaacctatacataatagaaacaaattatactta

SEQ ID NO: 90 - DNA, 308 bp, Artificial Sequence
  gBlock12-PV-3'TR-5'TR
cctatacataatagaaacaaattatacttattagtcagtcagaaacaactttggcacatatcaatattatgctctgctagcgatatctgtaaaacgacggccagttctagacttaagcttcatggtcatagctgtttcctgctcgagttaattaaccaacaagctcgtcatcgctttgcagaagagcagagaggatatgctcatcgtctaaagaactacccattttattatatattagtcacgatatctataacaagaaaatatatatataataagttatcacgtaagtagaacatgaaataacaata

SEQ ID NO: 91 - DNA, 315 bp, Artificial Sequence
  gBlock13-PV-3'TR-5'TR
atcacgtaagtagaacatgaaataacaatataattatcgtatgagttaaatcttaaaagtcacgtaaaagataatcatgcgtcattttgactcacgcggtcgttatagttcaaaatcagtgacacttaccgcattgacaagcacgcctcacgggagctccaagcggcgactgagatgtcctaaatgcacagcgacggattcgcgctatttagaaagagagagcaatatttcaagaatgcatgcgtcaattttacgcagactatctttctagggttaatacgtataatacatatgattcagctgcattaatgaatc

SEQ ID NO: 92 - DNA, 33 bp, Artificial Sequence
  primer pHL-PacI-rHBB-pA-IF-fw
gtatacctcgagttaaattcactcctcaggtgc

SEQ ID NO: 93 - DNA, 38 bp, Artificial Sequence
  primer pPV-PacI-rHBB-pA-IF-rev
cgagcttgttggttaattaagtcgagggatctccataa

SEQ ID NO: 94 - DNA, 19 bp, Artificial Sequence
  primer Luc2-NcoI-IF-Fwd
gcccccttcaccatggaag

SEQ ID NO: 95 - DNA, 20 bp, Artificial Sequence
  primer Luc2-V323I-fwd
cagcaaggagataggtgagg

SEQ ID NO: 96 - DNA, 20 bp, Artificial Sequence
  primer Luc2-V323I-rev
cctcacctatctccttgctg

SEQ ID NO: 97 - DNA, 27 bp, Artificial Sequence
  primer Luc2-SalI-IF-Rev
taatgcaaacgtcgacaaatcaaagac

SEQ ID NO: 98 - DNA, 22 bp, Artificial Sequence
  primer DMD-Ex45-SalI-IF-F
tctttgatttgtcgaccgtatc

SEQ ID NO: 99 - DNA, 19 bp, Artificial Sequence
  primer DMD-Ex45-SalI-IF-R
taatgcaaacgtcgacgcc

SEQ ID NO: 100 - DNA, 38 bp, Artificial Sequence
  primer HDMD-SR-1kbFrag-fwd
tctttgatttgtcgagggatatcttgatgggatgctcc

SEQ ID NO: 101 - DNA, 37 bp, Artificial Sequence
  primer HDMD-SR-1kbFrag-rev
taatgcaaacgtcgaaaaccactaactagccacaagt

SEQ ID NO: 102 - DNA, 35 bp, Artificial Sequence
  primer HDMD-SR-2kbFrag-fwd
tctttgatttgtcgaattgtgaggcaccgtgtcac

SEQ ID NO: 103 - DNA, 36 bp, Artificial Sequence
  primer HDMD-SR-2kbFrag-rev
taatgcaaacgtcgactctttggctcaagttcccct

SEQ ID NO: 104 - DNA, 37 bp, Artificial Sequence
  primer HDMD-SR-4kbFrag-fwd
tctttgatttgtcgagctgcagcattagtttatagca

SEQ ID NO: 105 - DNA, 35 bp, Artificial Sequence
  primer HDMD-SR-4kbFrag-rev
taatgcaaacgtcgaaactttggcaaggggtgtgt

SEQ ID NO: 106 - DNA, 1744 bp, Artificial Sequence
  Luc2(V323I)-hDMD-Ex45[-]
atggaagatgccaaaaacattaagaagggcccagcgccattctacccactcgaagacgggaccgccggcgagcagctgcacaaagccatgaagcgctacgccctggtgcccggcaccatcgcctttaccgacgcacatatcgaggtggacattacctacgccgagtacttcgagatgagcgttcggctggcagaagctatgaagcgctatgggctgaatacaaaccatcggatcgtggtgtgcagcgagaatagcttgcagttcttcatgcccgtgttgggtgccctgttcatcggtgtggctgtggccccagctaacgacatctacaacgagcgcgagctgctgaacagcatgggcatcagccagcccaccgtcgtattcgtgagcaagaaagggctgcaaaagatcctcaacgtgcaaaagaagctaccgatcatacaaaagatcatcatcatggatagcaagaccgactaccagggcttccaaagcatgtacaccttcgtgacttcccatttgccacccggcttcaacgagtacgacttcgtgcccgagagcttcgaccgggacaaaaccatcgccctgatcatgaacagtagtggcagtaccggattgcccaagggcgtagccctaccgcaccgcaccgcttgtgtccgattcagtcatgcccgcgaccccatcttcggcaaccagatcatccccgacaccgctatcctcagcgtggtgccatttcaccacggcttcggcatgttcaccacgctgggctacttgatctgcggctttcgggtcgtgctcatgtaccgcttcgaggaggagctattcttgcgcagcttgcaagactataagattcaatctgccctgctggtgcccacactatttagcttcttcgctaagagcactctcatcgacaagtacgacctaagcaacttgcacgagatcgccagcggcggggcgccgctcagcaaggagataggtgaggccgtggccaaacgcttccacctaccaggtaagtctttgatttgtcgacgtttgcattaacaaatagtttgagaactatgttggaaaaaaaaataacaattttattcttctttctccaggcatccgccagggctacggcctgacagaaacaaccagcgccattctgatcacccccgaaggggacgacaagcctggcgcagtaggcaaggtggtgcccttcttcgaggctaaggtggtggacttggacaccggtaagacactgggtgtgaaccagcgcggcgagctgtgcgtccgtggccccatgatcatgagcggctacgttaacaaccccgaggctacaaacgctctcatcgacaaggacggctggctgcacagcggcgacatcgcctactgggacgaggacgagcacttcttcatcgtggaccggctgaagagcctgatcaaatacaagggctaccaggtagccccagccgaactggagagcatcctgctgcaacaccccaacatcttcgacgccggggtcgccggcctgcccgacgacgatgccggcgagctgcccgccgcagtcgtcgtgctggaacacggtaaaaccatgaccgagaaggagatcgtggactatgtggccagccaggttacaaccgccaagaagctgcgcggtggtgttgtgttcgtggacgaggtgcctaaaggactgaccggcaagttggacgcccgcaagatccgcgagattctcattaaggccaagaagggcggcaagatcgccgtgtaa

SEQ ID NO: 107 - DNA, 2442 bp, Artificial Sequence
  Luc2(V323I)-hDMD-Ex45[+]
atggaagatgccaaaaacattaagaagggcccagcgccattctacccactcgaagacgggaccgccggcgagcagctgcacaaagccatgaagcgctacgccctggtgcccggcaccatcgcctttaccgacgcacatatcgaggtggacattacctacgccgagtacttcgagatgagcgttcggctggcagaagctatgaagcgctatgggctgaatacaaaccatcggatcgtggtgtgcagcgagaatagcttgcagttcttcatgcccgtgttgggtgccctgttcatcggtgtggctgtggccccagctaacgacatctacaacgagcgcgagctgctgaacagcatgggcatcagccagcccaccgtcgtattcgtgagcaagaaagggctgcaaaagatcctcaacgtgcaaaagaagctaccgatcatacaaaagatcatcatcatggatagcaagaccgactaccagggcttccaaagcatgtacaccttcgtgacttcccatttgccacccggcttcaacgagtacgacttcgtgcccgagagcttcgaccgggacaaaaccatcgccctgatcatgaacagtagtggcagtaccggattgcccaagggcgtagccctaccgcaccgcaccgcttgtgtccgattcagtcatgcccgcgaccccatcttcggcaaccagatcatccccgacaccgctatcctcagcgtggtgccatttcaccacggcttcggcatgttcaccacgctgggctacttgatctgcggctttcgggtcgtgctcatgtaccgcttcgaggaggagctattcttgcgcagcttgcaagactataagattcaatctgccctgctggtgcccacactatttagcttcttcgctaagagcactctcatcgacaagtacgacctaagcaacttgcacgagatcgccagcggcggggcgccgctcagcaaggagataggtgaggccgtggccaaacgcttccacctaccaggtaagtctttgatttgtcgaccgtatccacgatcactaagaaacccaaatactttgttcatgtttaaattttacaacatttcatagactattaaacatggaacatccttgtggggacaagaaatcgaatttgctcttgaaaaggtttccaactaattgatttgtaggacattataacatcctctagctgacaagcttacaaaaataaaaactggagctaaccgagagggtgcttttttccctgacacataaaaggtgtctttctgtcttgtatcctttggatatgggcatgtcagtttcatagggaaattttcacatggagcttttgtatttctttctttgccagtacaactgcatgtggtagcacactgtttaatcttttctcaaataaaaagacatggggcttcatttttgttttgcctttttggtatcttacaggaactccaggatggcattgggcagcggcaaactgttgtcagaacattgaatgcaactggggaagaaataattcagcaatcctcaaaaacagatgccagtattctacaggaaaaattgggaagcctgaatctgcggtggcaggaggtctgcaaacagctgtcagacagaaaaaagaggtagggcgacagatctaataggaatgaaaacattttagcagactttttaagctttctttagaagaatatttcatgagagattataagcagggtgaaaggcgtcgacgtttgcattaacaaatagtttgagaactatgttggaaaaaaaaataacaattttattcttctttctccaggcatccgccagggctacggcctgacagaaacaaccagcgccattctgatcacccccgaaggggacgacaagcctggcgcagtaggcaaggtggtgcccttcttcgaggctaaggtggtggacttggacaccggtaagacactgggtgtgaaccagcgcggcgagctgtgcgtccgtggccccatgatcatgagcggctacgttaacaaccccgaggctacaaacgctctcatcgacaaggacggctggctgcacagcggcgacatcgcctactgggacgaggacgagcacttcttcatcgtggaccggctgaagagcctgatcaaatacaagggctaccaggtagccccagccgaactggagagcatcctgctgcaacaccccaacatcttcgacgccggggtcgccggcctgcccgacgacgatgccggcgagctgcccgccgcagtcgtcgtgctggaacacggtaaaaccatgaccgagaaggagatcgtggactatgtggccagccaggttacaaccgccaagaagctgcgcggtggtgttgtgttcgtggacgaggtgcctaaaggactgaccggcaagttggacgcccgcaagatccgcgagattctcattaaggccaagaagggcggcaagatcgccgtgtaa

SEQ ID NO: 108 - DNA, 2676 bp, Artificial Sequence
  Luc2(V323I)-hDMD-Ex45[+](1kb)
atggaagatgccaaaaacattaagaagggcccagcgccattctacccactcgaagacgggaccgccggcgagcagctgcacaaagccatgaagcgctacgccctggtgcccggcaccatcgcctttaccgacgcacatatcgaggtggacattacctacgccgagtacttcgagatgagcgttcggctggcagaagctatgaagcgctatgggctgaatacaaaccatcggatcgtggtgtgcagcgagaatagcttgcagttcttcatgcccgtgttgggtgccctgttcatcggtgtggctgtggccccagctaacgacatctacaacgagcgcgagctgctgaacagcatgggcatcagccagcccaccgtcgtattcgtgagcaagaaagggctgcaaaagatcctcaacgtgcaaaagaagctaccgatcatacaaaagatcatcatcatggatagcaagaccgactaccagggcttccaaagcatgtacaccttcgtgacttcccatttgccacccggcttcaacgagtacgacttcgtgcccgagagcttcgaccgggacaaaaccatcgccctgatcatgaacagtagtggcagtaccggattgcccaagggcgtagccctaccgcaccgcaccgcttgtgtccgattcagtcatgcccgcgaccccatcttcggcaaccagatcatccccgacaccgctatcctcagcgtggtgccatttcaccacggcttcggcatgttcaccacgctgggctacttgatctgcggctttcgggtcgtgctcatgtaccgcttcgaggaggagctattcttgcgcagcttgcaagactataagattcaatctgccctgctggtgcccacactatttagcttcttcgctaagagcactctcatcgacaagtacgacctaagcaacttgcacgagatcgccagcggcggggcgccgctcagcaaggagataggtgaggccgtggccaaacgcttccacctaccaggtaagtctttgatttgtcgaagcacgcatttggctttctgtgccttcaatacattccaagggaaatttaaatgatgattgaatttgacagtaacctttttgaggttttgttttccccattaaacttgtacctctttggctcaagttccccttcaagaatgtattcacaaatgtggtgaaactagaggtaagtgacactatcactttttttagcttcatagtcatattcatagctatttttaaaactaagcaaagatctgtctttcctacaaaacaatcatttataattgctttctaaaatcttcttgaaaaacaactgagattcagcttgttgaagttaaaatatattgaagatattcacctttaagcaatcatgggtgatttttaaagcaaacttcaagtttaaaatagcagaaaaccactaactagccacaagtatatattttagtatatgaaaaaaagaaataaaaaatttctttactgctgttgattaatggttgataggttctttaatgttagtgcctttcaccctgcttataatctctcatgaaatattcttctaaagaaagcttaaaaagtctgctaaaatgttttcattcctattagatctgtcgccctacctcttttttctgtctgacagctgtttgcagacctcctgccaccgcagattcaggcttcccaatttttcctgtagaatactggcatctgtttttgaggattgctgaattatttcttccccagttgcattcaatgttctgacaacagtttgccgctgcccaatgccatcctggagttcctgtaagataccaaaaaggcaaaacaaaaatgaagccccatgtctttttatttgagaaaagattaaacagtgtgctaccacatgcagttgtactggcaaagaaagaaatacaaaagctccatgtgaaaatttccctatgaaactgacatgccctcgacgtttgcattaacaaatagtttgagaactatgttggaaaaaaaaataacaattttattcttctttctccaggcatccgccagggctacggcctgacagaaacaaccagcgccattctgatcacccccgaaggggacgacaagcctggcgcagtaggcaaggtggtgcccttcttcgaggctaaggtggtggacttggacaccggtaagacactgggtgtgaaccagcgcggcgagctgtgcgtccgtggccccatgatcatgagcggctacgttaacaaccccgaggctacaaacgctctcatcgacaaggacggctggctgcacagcggcgacatcgcctactgggacgaggacgagcacttcttcatcgtggaccggctgaagagcctgatcaaatacaagggctaccaggtagccccagccgaactggagagcatcctgctgcaacaccccaacatcttcgacgccggggtcgccggcctgcccgacgacgatgccggcgagctgcccgccgcagtcgtcgtgctggaacacggtaaaaccatgaccgagaaggagatcgtggactatgtggccagccaggttacaaccgccaagaagctgcgcggtggtgttgtgttcgtggacgaggtgcctaaaggactgaccggcaagttggacgcccgcaagatccgcgagattctcattaaggccaagaagggcggcaagatcgccgtgtaa

SEQ ID NO: 109 - DNA, 3651 bp, Artificial Sequence
  Luc2(V323I)-hDMD-Ex45[+](2kb)
atggaagatgccaaaaacattaagaagggcccagcgccattctacccactcgaagacgggaccgccggcgagcagctgcacaaagccatgaagcgctacgccctggtgcccggcaccatcgcctttaccgacgcacatatcgaggtggacattacctacgccgagtacttcgagatgagcgttcggctggcagaagctatgaagcgctatgggctgaatacaaaccatcggatcgtggtgtgcagcgagaatagcttgcagttcttcatgcccgtgttgggtgccctgttcatcggtgtggctgtggccccagctaacgacatctacaacgagcgcgagctgctgaacagcatgggcatcagccagcccaccgtcgtattcgtgagcaagaaagggctgcaaaagatcctcaacgtgcaaaagaagctaccgatcatacaaaagatcatcatcatggatagcaagaccgactaccagggcttccaaagcatgtacaccttcgtgacttcccatttgccacccggcttcaacgagtacgacttcgtgcccgagagcttcgaccgggacaaaaccatcgccctgatcatgaacagtagtggcagtaccggattgcccaagggcgtagccctaccgcaccgcaccgcttgtgtccgattcagtcatgcccgcgaccccatcttcggcaaccagatcatccccgacaccgctatcctcagcgtggtgccatttcaccacggcttcggcatgttcaccacgctgggctacttgatctgcggctttcgggtcgtgctcatgtaccgcttcgaggaggagctattcttgcgcagcttgcaagactataagattcaatctgccctgctggtgcccacactatttagcttcttcgctaagagcactctcatcgacaagtacgacctaagcaacttgcacgagatcgccagcggcggggcgccgctcagcaaggagataggtgaggccgtggccaaacgcttccacctaccaggtaagtctttgatttgtcgatctttaactttggcaaggggtgtgtgtgtgtgtgtgtgtgtgtgtgtgtgtgtgtgtgtgtgtgtgtgtgtgtgtgtttaggtcaactaatgtgtttattttgtacaaaatatgaattgtatctactttctgaataatgtaacatgaataaagagggaaagaggaggtgggcaaagacaactgacataattccaaaatcttctttttaatacatcttaacgaaagatattcatcaatgagttgttctagcttcctgaatattaaaatccacctattatgtggatgatgggtgggatgcaagagcttggcaaaagaacgaagttttcattgttcataacaatagtctcatttggtaaataaaggccaagtcttcctttacgaaacaagacacattaacatcaacaactggaagcataatacaaaatcccatttataaactctctaggctttccaactgcagcagcacgcatttggctttctgtgccttcaatacattccaagggaaatttaaatgatgattgaatttgacagtaacctttttgaggttttgttttccccattaaacttgtacctctttggctcaagttccccttcaagaatgtattcacaaatgtggtgaaactagaggtaagtgacactatcactttttttagcttcatagtcatattcatagctatttttaaaactaagcaaagatctgtctttcctacaaaacaatcatttataattgctttctaaaatcttcttgaaaaacaactgagattcagcttgttgaagttaaaatatattgaagatattcacctttaagcaatcatgggtgatttttaaagcaaacttcaagtttaaaatagcagaaaaccactaactagccacaagtatatattttagtatatgaaaaaaagaaataaaaaatttctttactgctgttgattaatggttgataggttctttaatgttagtgcctttcaccctgcttataatctctcatgaaatattcttctaaagaaagcttaaaaagtctgctaaaatgttttcattcctattagatctgtcgccctacctcttttttctgtctgacagctgtttgcagacctcctgccaccgcagattcaggcttcccaatttttcctgtagaatactggcatctgtttttgaggattgctgaattatttcttccccagttgcattcaatgttctgacaacagtttgccgctgcccaatgccatcctggagttcctgtaagataccaaaaaggcaaaacaaaaatgaagccccatgtctttttatttgagaaaagattaaacagtgtgctaccacatgcagttgtactggcaaagaaagaaatacaaaagctccatgtgaaaatttccctatgaaactgacatgcccatatccaaaggatacaagacagaaagacaccttttatgtgtcagggaaaaaagcaccctctcggttagctccagtttttatttttgtaagcttgtcagctagaggatgttataatgtcctacaaatcaattagttggaaaccttttcaagagcaaattcgatttcttgtccccacaaggatgttccatgtttaatagtctatgaaatgttgtaaaatttaaacatgaacaaagtatttgggtttcttagtgatcgtggatacgagaggtgaaaaagaacaaacataggttagtcacagtattaaaaaaaaactctagagatatttaaataaaattaattgctatattagaagaaaattcatttcaaattctgtctgcgtcaatgtattttgcattagaagccacaaaaaactgagaattaattgctttcaggagcatcccatcaagatatccctaagctacagtaataaattttaaaataatctatagtcaccagagcatttttatgattgtcatcgacgtttgcattaacaaatagtttgagaactatgttggaaaaaaaaataacaattttattcttctttctccaggcatccgccagggctacggcctgacagaaacaaccagcgccattctgatcacccccgaaggggacgacaagcctggcgcagtaggcaaggtggtgcccttcttcgaggctaaggtggtggacttggacaccggtaagacactgggtgtgaaccagcgcggcgagctgtgcgtccgtggccccatgatcatgagcggctacgttaacaaccccgaggctacaaacgctctcatcgacaaggacggctggctgcacagcggcgacatcgcctactgggacgaggacgagcacttcttcatcgtggaccggctgaagagcctgatcaaatacaagggctaccaggtagccccagccgaactggagagcatcctgctgcaacaccccaacatcttcgacgccggggtcgccggcctgcccgacgacgatgccggcgagctgcccgccgcagtcgtcgtgctggaacacggtaaaaccatgaccgagaaggagatcgtggactatgtggccagccaggttacaaccgccaagaagctgcgcggtggtgttgtgttcgtggacgaggtgcctaaaggactgaccggcaagttggacgcccgcaagatccgcgagattctcattaaggccaagaagggcggcaagatcgccgtgtaa

SEQ ID NO: 110 - DNA, 5709 bp, Artificial Sequence
  Luc2(V323I)-hDMD-Ex45[+](4kb)
atggaagatgccaaaaacattaagaagggcccagcgccattctacccactcgaagacgggaccgccggcgagcagctgcacaaagccatgaagcgctacgccctggtgcccggcaccatcgcctttaccgacgcacatatcgaggtggacattacctacgccgagtacttcgagatgagcgttcggctggcagaagctatgaagcgctatgggctgaatacaaaccatcggatcgtggtgtgcagcgagaatagcttgcagttcttcatgcccgtgttgggtgccctgttcatcggtgtggctgtggccccagctaacgacatctacaacgagcgcgagctgctgaacagcatgggcatcagccagcccaccgtcgtattcgtgagcaagaaagggctgcaaaagatcctcaacgtgcaaaagaagctaccgatcatacaaaagatcatcatcatggatagcaagaccgactaccagggcttccaaagcatgtacaccttcgtgacttcccatttgccacccggcttcaacgagtacgacttcgtgcccgagagcttcgaccgggacaaaaccatcgccctgatcatgaacagtagtggcagtaccggattgcccaagggcgtagccctaccgcaccgcaccgcttgtgtccgattcagtcatgcccgcgaccccatcttcggcaaccagatcatccccgacaccgctatcctcagcgtggtgccatttcaccacggcttcggcatgttcaccacgctgggctacttgatctgcggctttcgggtcgtgctcatgtaccgcttcgaggaggagctattcttgcgcagcttgcaagactataagattcaatctgccctgctggtgcccacactatttagcttcttcgctaagagcactctcatcgacaagtacgacctaagcaacttgcacgagatcgccagcggcggggcgccgctcagcaaggagataggtgaggccgtggccaaacgcttccacctaccaggtaagtctttgatttgtcgatttgcaactacagggctccatatagacatctagcttgaatttatacactttctttcattgatgtccctggactaaaaaatgttaaatatttctaaccgctgtacttaaagtccattacaaacgaagactactgttgttaagttgaataggcatcttatatatttttcaccggtgcaataaataacttctattcccttctaacatctgcttgcgttgcactgagagtacactattgattagcaataggttcgtgattacagcccttctataattaattgttaggttaacatattattcataaaatattattttattaatttttacttgatttgctactggatgcttagaaatagctatgagtatattggtagaaccagtacttatattttattacatttttacatttcataaaatttaagtgatataaaaatcctgaggaagtatgccacaaaagtggtctcagtggaaatttaaatatgttaacatttatttttaaaatgtagcgtgaaatagacaactttaaaagctcagcttaaaaaaaaaactcaaggaagctgaacttgactttttaaagcactgaagtgcaatatttaatgtaggtcaacatgtttaaatgggaaaatttttttcctaattacagccaaatccctagctgtaattaacttaaaatttgtatactatttcacaacagagtcagcatataccactttcttataaaattagaaagatctaaaattttagagcttatttggtgaaacaggcatattgctacatctttgtttataaattataatgtgcctttagagcccaataacagataacaagattttgaaaattcaggtgaattagagttatcagagggaatgttaatacactctattcaaatactatatgagtaagacatttaaaataggaaacaatactttatatattatagaaaaataatcttccagtcgatttaatccactttatgaattctctccgtatatatatatttatagtatggtattcaatttttttaattttctcatttcttaccatcttaatttggattagattgagcctagttcagaaatgacattatacaggtttatacctgttcatagtataagcacatcagttatctaaataataaaatacttgtatgattaagagaagaatttcaatctgggaaaaaagtatatgacttacctaaggaagtagtttaactacaaagtttagttctttattttatctatctataatcaagaagattttcaaaaccaagacttaattattcaaaatatcttttgatgaggctataattctttaactttggcaaggggtgtgtgtgtgtgtgtgtgtgtgtgtgtgtgtgtgtgtgtgtgtgtgtgtgtgtgtgtttaggtcaactaatgtgtttattttgtacaaaatatgaattgtatctactttctgaataatgtaacatgaataaagagggaaagaggaggtgggcaaagacaactgacataattccaaaatcttctttttaatacatcttaacgaaagatattcatcaatgagttgttctagcttcctgaatattaaaatccacctattatgtggatgatgggtgggatgcaagagcttggcaaaagaacgaagttttcattgttcataacaatagtctcatttggtaaataaaggccaagtcttcctttacgaaacaagacacattaacatcaacaactggaagcataatacaaaatcccatttataaactctctaggctttccaactgcagcagcacgcatttggctttctgtgccttcaatacattccaagggaaatttaaatgatgattgaatttgacagtaacctttttgaggttttgttttccccattaaacttgtacctctttggctcaagttccccttcaagaatgtattcacaaatgtggtgaaactagaggtaagtgacactatcactttttttagcttcatagtcatattcatagctatttttaaaactaagcaaagatctgtctttcctacaaaacaatcatttataattgctttctaaaatcttcttgaaaaacaactgagattcagcttgttgaagttaaaatatattgaagatattcacctttaagcaatcatgggtgatttttaaagcaaacttcaagtttaaaatagcagaaaaccactaactagccacaagtatatattttagtatatgaaaaaaagaaataaaaaatttctttactgctgttgattaatggttgataggttctttaatgttagtgcctttcaccctgcttataatctctcatgaaatattcttctaaagaaagcttaaaaagtctgctaaaatgttttcattcctattagatctgtcgccctacctcttttttctgtctgacagctgtttgcagacctcctgccaccgcagattcaggcttcccaatttttcctgtagaatactggcatctgtttttgaggattgctgaattatttcttccccagttgcattcaatgttctgacaacagtttgccgctgcccaatgccatcctggagttcctgtaagataccaaaaaggcaaaacaaaaatgaagccccatgtctttttatttgagaaaagattaaacagtgtgctaccacatgcagttgtactggcaaagaaagaaatacaaaagctccatgtgaaaatttccctatgaaactgacatgcccatatccaaaggatacaagacagaaagacaccttttatgtgtcagggaaaaaagcaccctctcggttagctccagtttttatttttgtaagcttgtcagctagaggatgttataatgtcctacaaatcaattagttggaaaccttttcaagagcaaattcgatttcttgtccccacaaggatgttccatgtttaatagtctatgaaatgttgtaaaatttaaacatgaacaaagtatttgggtttcttagtgatcgtggatacgagaggtgaaaaagaacaaacataggttagtcacagtattaaaaaaaaactctagagatatttaaataaaattaattgctatattagaagaaaattcatttcaaattctgtctgcgtcaatgtattttgcattagaagccacaaaaaactgagaattaattgctttcaggagcatcccatcaagatatccctaagctacagtaataaattttaaaataatctatagtcaccagagcatttttatgattgtcaagcttaaatattgtttacttttttcctgaatgaaattttaagagtaaagtatcagaaaaatagctcaattgaaaaggagaatattacaaccaagtacacacaaaaacaaaaatgctttttaccattaaataaaaatggcaattacgttctatttaactttttaaaaaagataatctagaatttgtaaggccattaaaataacatattaactaaatacgaaccttagaaaatgaaataatatctgagaacttgaggtacctaccgtatttaaatctgaatgactcaaatccttatgtcactgacagaataatgtgcgtatgtagaaaactctcctaatagatgtgattcatattctctaatatttttgtattctcctactccttgacacaatagcaagctgacagtagaccccagtacatgcttcctaaatgaaggaaggaatgcatgttttctgagactgaggtaaagctcccttagactctcgtttcacatacatttcttggcttttttctttttctacattcaagcaaaattattttcgaatactggaaattttggtagcatacagttagcaattaaaatactctgtaaatcagcaaaccggtgacacggtgcctcacaatgaatataaaactatgcacagttactgaactattcacaagctgtcctggccatactctcttgaatgcccatgagatgtgctctagtaaacatgtgatatttccttgtaactagttggctttgctccattgctcgacgtttgcattaacaaatagtttgagaactatgttggaaaaaaaaataacaattttattcttctttctccaggcatccgccagggctacggcctgacagaaacaaccagcgccattctgatcacccccgaaggggacgacaagcctggcgcagtaggcaaggtggtgcccttcttcgaggctaaggtggtggacttggacaccggtaagacactgggtgtgaaccagcgcggcgagctgtgcgtccgtggccccatgatcatgagcggctacgttaacaaccccgaggctacaaacgctctcatcgacaaggacggctggctgcacagcggcgacatcgcctactgggacgaggacgagcacttcttcatcgtggaccggctgaagagcctgatcaaatacaagggctaccaggtagccccagccgaactggagagcatcctgctgcaacaccccaacatcttcgacgccggggtcgccggcctgcccgacgacgatgccggcgagctgcccgccgcagtcgtcgtgctggaacacggtaaaaccatgaccgagaaggagatcgtggactatgtggccagccaggttacaaccgccaagaagctgcgcggtggtgttgtgttcgtggacgaggtgcctaaaggactgaccggcaagttggacgcccgcaagatccgcgagattctcattaaggccaagaagggcggcaagatcgccgtgtaa

SEQ ID NO: 111 - protein, 22 aa, Artificial Sequence
  artificial peptide
ASGGAPLSKEVGEAVAKRFHLP

SEQ ID NO: 112 - protein, 48 aa, Artificial Sequence
  artificial peptide
GIRQGYGLTETTSAILITPEGDDKPGAVGKVVPFFEAKVVDLDTGKTL

SEQ ID NO: 113 - DNA, 29 bp, Artificial Sequence
  artificial sequence
ccgctcagcaaggaggtaggtgaggccgt

SEQ ID NO: 114 - DNA, 15 bp, Artificial Sequence
  artificial sequence
aaggaggtaggtgag

SEQ ID NO: 115 - protein, 5 aa, Artificial Sequence
  artificial sequence
KEVGE

SEQ ID NO: 116 - DNA, 15 bp, Artificial Sequence
  artificial sequence
aaggagataggtgag

SEQ ID NO: 117 - protein, 5 aa, Artificial Sequence
  artificial sequence
KEIGE

SEQ ID NO: 118 - DNA, 79 bp, Artificial Sequence
  artificial sequence
gttttgcctttttggtatcttacaggaactccaggatggcattgggcagcggcaaactgttgtcagaacattgaatgca

SEQ ID NO: 119 - DNA, 79 bp, Artificial Sequence
  artificial sequence
tgcattcaatgttctgacaacagtttgccgctgcccaatgccatcctggagttcctgtaagataccaaaaaggcaaaac

SEQ ID NO: 120 - DNA, 23 bp, Artificial Sequence
  artificial sequence
tggtatcttacaggaactccagg

SEQ ID NO: 121 - DNA, 23 bp, Artificial Sequence
  artificial sequence
atcttacaggaactccaggatgg

SEQ ID NO: 122 - DNA, 23 bp, Artificial Sequence
  artificial sequence
caggaactccaggatggcattgg

SEQ ID NO: 123 - DNA, 23 bp, Artificial Sequence
  artificial sequence
tccaggatggcattgggcagcgg

SEQ ID NO: 124 - DNA, 23 bp, Artificial Sequence
  artificial sequence
gttcctgtaagataccaaaaagg

SEQ ID NO: 125 - DNA, 62 bp, Artificial Sequence
  artificial sequence
ttgttttgcctttttggtatcttacaggaactccaggatggcattgggcagcggcaaactgt

SEQ ID NO: 126 - DNA, 73 bp, Artificial Sequence
  artificial sequence
ttttgcctttttggtatcttacaggaactccaggatggcattgggcagcggcaaactgttgtcagaacattga

SEQ ID NO: 127 - DNA, 73 bp, Artificial Sequence
  artificial sequence
tcaatgttctgacaacagtttgccgctgcccaatgccatcctggagttcctgtaagataccaaaaaggcaaaa

SEQ ID NO: 128 - DNA, 23 bp, Artificial Sequence
  artificial sequence
tggtatcttacaggaactccagg

SEQ ID NO: 129 - DNA, 23 bp, Artificial Sequence
  artificial sequence
tccaggatggcattgggcagcgg

SEQ ID NO: 130 - DNA, 23 bp, Artificial Sequence
  artificial sequence
gttcctgtaagataccaaaaagg

SEQ ID NO: 131 - DNA, 29 bp, Artificial Sequence
  artificial sequence
cttacaggaactccaggatggcattgggc

SEQ ID NO: 132 - DNA, 29 bp, Artificial Sequence
  artificial sequence
tttgccgctgcccaatgccatcctggagt

SEQ ID NO: 133 - DNA, 24 bp, Artificial Sequence
  artificial sequence
tttttggtatcttacaggaactcc

SEQ ID NO: 134 - DNA, 24 bp, Artificial Sequence
  artificial sequence
ttttggtatcttacaggaactcca

SEQ ID NO: 135 - DNA, 24 bp, Artificial Sequence
  artificial sequence
tttggtatcttacaggaactccag

SEQ ID NO: 136 - DNA, 24 bp, Artificial Sequence
  artificial sequence
tttgccgctgcccaatgccatcct

SEQ ID NO: 137 - DNA, 23 bp, Artificial Sequence
  artificial sequence
ggtcctaccgtaacccgtcgccg

SEQ ID NO: 138 - DNA, 23 bp, Artificial Sequence
  artificial sequence
ggtcataagatgtcctttttaac

SEQ ID NO: 139 - DNA, 23 bp, Artificial Sequence
  artificial sequence
ggaaaaaccatagaatgtccttg

SEQ ID NO: 140 - DNA, 23 bp, Artificial Sequence
  artificial sequence
ggagtttttgtctacggtcataa

SEQ ID NO: 141 - DNA, 23 bp, Artificial Sequence
  artificial sequence
ggacttagacgccaccgtcctcc

SEQ ID NO: 142 - DNA, 247 bp, Artificial Sequence
  artificial sequence
catggggcttcatttttgttttgcctttttggtatcttacaggaactccaggatggcattgggcagcggcaaactgttgtcagaacattgaatgcaactggggaagaaataattcagcaatcctcaaaaacagatgccagtattctacaggaaaaattgggaagcctgaatctgcggtggcaggaggtctgcaaacagctgtcagacagaaaaaagaggtagggcgacagatctaataggaatgaaa

SEQ ID NO: 143 - DNA, 247 bp, Artificial Sequence
  artificial sequence
tttcattcctattagatctgtcgccctacctcttttttctgtctgacagctgtttgcagacctcctgccaccgcagattcaggcttcccaatttttcctgtagaatactggcatctgtttttgaggattgctgaattatttcttccccagttgcattcaatgttctgacaacagtttgccgctgcccaatgccatcctggagttcctgtaagataccaaaaaggcaaaacaaaaatgaagccccatg

SEQ ID NO: 144 - DNA, 23 bp, Artificial Sequence
  artificial sequence
tcatttttgttttgcctttttgg

SEQ ID NO: 145 - DNA, 23 bp, Artificial Sequence
  artificial sequence
gtcagaacattgaatgcaactgg

SEQ ID NO: 146 - DNA, 23 bp, Artificial Sequence
  artificial sequence
aacagatgccagtattctacagg

SEQ ID NO: 147 - DNA, 23 bp, Artificial Sequence
  artificial sequence
agctgtcagacagaaaaaagagg

SEQ ID NO: 148 - DNA, 23 bp, Artificial Sequence
  artificial sequence
ttgcctttttggtatcttacagg

SEQ ID NO: 149 - DNA, 23 bp, Artificial Sequence
  artificial sequence
tcagaacattgaatgcaactggg

SEQ ID NO: 150 - DNA, 23 bp, Artificial Sequence
  artificial sequence
cagtattctacaggaaaaattgg

SEQ ID NO: 151 - DNA, 23 bp, Artificial Sequence
  artificial sequence
gtcagacagaaaaaagaggtagg

SEQ ID NO: 152 - DNA, 23 bp, Artificial Sequence
  artificial sequence
tggtatcttacaggaactccagg

SEQ ID NO: 153 - DNA, 23 bp, Artificial Sequence
  artificial sequence
cagaacattgaatgcaactgggg

SEQ ID NO: 154 - DNA, 23 bp, Artificial Sequence
  artificial sequence
agtattctacaggaaaaattggg

SEQ ID NO: 155 - DNA, 23 bp, Artificial Sequence
  artificial sequence
tcagacagaaaaaagaggtaggg

SEQ ID NO: 156 - DNA, 23 bp, Artificial Sequence
  artificial sequence
atcttacaggaactccaggatgg

SEQ ID NO: 157 - DNA, 23 bp, Artificial Sequence
  artificial sequence
aattgggaagcctgaatctgcgg

SEQ ID NO: 158 - DNA, 23 bp, Artificial Sequence
  artificial sequence
ggtagggcgacagatctaatagg

SEQ ID NO: 159 - DNA, 23 bp, Artificial Sequence
  artificial sequence
caggaactccaggatggcattgg

SEQ ID NO: 160 - DNA, 23 bp, Artificial Sequence
  artificial sequence
tgggaagcctgaatctgcggtgg

SEQ ID NO: 161 - DNA, 23 bp, Artificial Sequence
  artificial sequence
aggaactccaggatggcattggg

SEQ ID NO: 162 - DNA, 23 bp, Artificial Sequence
  artificial sequence
aagcctgaatctgcggtggcagg

SEQ ID NO: 163 - DNA, 23 bp, Artificial Sequence
  artificial sequence
tccaggatggcattgggcagcgg

SEQ ID NO: 164 - DNA, 23 bp, Artificial Sequence
  artificial sequence
cctgaatctgcggtggcaggagg

SEQ ID NO: 165 - DNA, 23 bp, Artificial Sequence
  artificial sequence
tggtatcttacaggaactccagg

SEQ ID NO: 166 - DNA, 20 bp, Artificial Sequence
  artificial sequence
gggtatcttacaggaactcc

SEQ ID NO: 167 - DNA, 23 bp, Artificial Sequence
  artificial sequence
atcttacaggaactccaggatgg

SEQ ID NO: 168 - DNA, 20 bp, Artificial Sequence
  artificial sequence
gtcttacaggaactccagga

SEQ ID NO: 169 - DNA, 23 bp, Artificial Sequence
  artificial sequence
caggaactccaggatggcattgg

SEQ ID NO: 170 - DNA, 20 bp, Artificial Sequence
  artificial sequence
gaggaactccaggatggcat

SEQ ID NO: 171 - DNA, 23 bp, Artificial Sequence
  artificial sequence
tccaggatggcattgggcagcgg

SEQ ID NO: 172 - DNA, 20 bp, Artificial Sequence
  artificial sequence
gccaggatggcattgggcag

SEQ ID NO: 173 - DNA, 23 bp, Artificial Sequence
  artificial sequence
gttcctgtaagataccaaaaagg

SEQ ID NO: 174 - DNA, 20 bp, Artificial Sequence
  artificial sequence
gttcctgtaagataccaaaa

SEQ ID NO: 175 - DNA, 23 bp, Artificial Sequence
  artificial sequence
tcatttttgttttgcctttttgg

SEQ ID NO: 176 - DNA, 20 bp, Artificial Sequence
  artificial sequence
acatttttgttttgcctttt

SEQ ID NO: 177 - DNA, 23 bp, Artificial Sequence
  artificial sequence
ttgcctttttggtatcttacagg

SEQ ID NO: 178 - DNA, 20 bp, Artificial Sequence
  artificial sequence
atgcctttttggtatcttac

SEQ ID NO: 179 - DNA, 23 bp, Artificial Sequence
  artificial sequence
aggaactccaggatggcattggg

SEQ ID NO: 180 - DNA, 20 bp, Artificial Sequence
  artificial sequence
aggaactccaggatggcatt

SEQ ID NO: 181 - DNA, 23 bp, Artificial Sequence
  artificial sequence
gccgctgcccaatgccatcctgg

SEQ ID NO: 182 - DNA, 20 bp, Artificial Sequence
  artificial sequence
gccgctgcccaatgccatcc

SEQ ID NO: 183 - DNA, 23 bp, Artificial Sequence
  artificial sequence
gtcagaacattgaatgcaactgg

SEQ ID NO: 184 - DNA, 20 bp, Artificial Sequence
  artificial sequence
gtcagaacattgaatgcaac

SEQ ID NO: 185 - DNA, 23 bp, Artificial Sequence
  artificial sequence
tcagaacattgaatgcaactggg

SEQ ID NO: 186 - DNA, 20 bp, Artificial Sequence
  artificial sequence
acagaacattgaatgcaact

SEQ ID NO: 187 - DNA, 23 bp, Artificial Sequence
  artificial sequence
cagaacattgaatgcaactgggg

SEQ ID NO: 188 - DNA, 20 bp, Artificial Sequence
  artificial sequence
gagaacattgaatgcaactg

SEQ ID NO: 189 - DNA, 23 bp, Artificial Sequence
  artificial sequence
aatactggcatctgtttttgagg

SEQ ID NO: 190 - DNA, 20 bp, Artificial Sequence
  artificial sequence
aatactggcatctgtttttg

SEQ ID NO: 191 - DNA, 23 bp, Artificial Sequence
  artificial sequence
aacagatgccagtattctacagg

SEQ ID NO: 192 - DNA, 20 bp, Artificial Sequence
  artificial sequence
aacagatgccagtattctac

SEQ ID NO: 193 - DNA, 23 bp, Artificial Sequence
  artificial sequence
caatttttcctgtagaatactgg

SEQ ID NO: 194 - DNA, 20 bp, Artificial Sequence
  artificial sequence
gaatttttcctgtagaatac

SEQ ID NO: 195 - DNA, 23 bp, Artificial Sequence
  artificial sequence
cagtattctacaggaaaaattgg

SEQ ID NO: 196 - DNA, 20 bp, Artificial Sequence
  artificial sequence
gagtattctacaggaaaaat

SEQ ID NO: 197 - DNA, 23 bp, Artificial Sequence
  artificial sequence
agtattctacaggaaaaattggg

SEQ ID NO: 198 - DNA, 20 bp, Artificial Sequence
  artificial sequence
agtattctacaggaaaaatt

SEQ ID NO: 199 - DNA, 23 bp, Artificial Sequence
  artificial sequence
aattgggaagcctgaatctgcgg

SEQ ID NO: 200 - DNA, 20 bp, Artificial Sequence
  artificial sequence
aattgggaagcctgaatctg

SEQ ID NO: 201 - DNA, 23 bp, Artificial Sequence
  artificial sequence
tgggaagcctgaatctgcggtgg

SEQ ID NO: 202 - DNA, 20 bp, Artificial Sequence
  artificial sequence
agggaagcctgaatctgcgg

SEQ ID NO: 203 - DNA, 23 bp, Artificial Sequence
  artificial sequence
aagcctgaatctgcggtggcagg

SEQ ID NO: 204 - DNA, 20 bp, Artificial Sequence
  artificial sequence
aagcctgaatctgcggtggc

SEQ ID NO: 205 - DNA, 23 bp, Artificial Sequence
  artificial sequence
cctgaatctgcggtggcaggagg

SEQ ID NO: 206 - DNA, 20 bp, Artificial Sequence
  artificial sequence
gctgaatctgcggtggcagg

SEQ ID NO: 207 - DNA, 23 bp, Artificial Sequence
  artificial sequence
cctcctgccaccgcagattcagg

SEQ ID NO: 208 - DNA, 20 bp, Artificial Sequence
  artificial sequence
gctcctgccaccgcagattc

SEQ ID NO: 209 - DNA, 23 bp, Artificial Sequence
  artificial sequence
agctgtcagacagaaaaaagagg

SEQ ID NO: 210 - DNA, 20 bp, Artificial Sequence
  artificial sequence
agctgtcagacagaaaaaag

SEQ ID NO: 211 - DNA, 23 bp, Artificial Sequence
  artificial sequence
gtcagacagaaaaaagaggtagg

SEQ ID NO: 212 - DNA, 20 bp, Artificial Sequence
  artificial sequence
gtcagacagaaaaaagaggt

SEQ ID NO: 213 - DNA, 23 bp, Artificial Sequence
  artificial sequence
tcagacagaaaaaagaggtaggg

SEQ ID NO: 214 - DNA, 20 bp, Artificial Sequence
  artificial sequence
acagacagaaaaaagaggta

SEQ ID NO: 215 - DNA, 23 bp, Artificial Sequence
  artificial sequence
ggtagggcgacagatctaatagg

SEQ ID NO: 216 - DNA, 20 bp, Artificial Sequence
  artificial sequence
ggtagggcgacagatctaat

SEQ ID NO: 217 - protein, 7 aa, Artificial Sequence
  NLS
PKKKRKV

SEQ ID NO: 218 - protein, 16 aa, Artificial Sequence
  NLS
KRPAATKKAGQAKKKK

SEQ ID NO: 219 - protein, 27 aa, Artificial Sequence
  HA
YPYDVPDYAYPYDVPDYAYPYDVPDYA